European Patent Specification EP 4 006 153 B1, published July 3, 2024. Title: ENHANCED IMMUNE CELLS USING DUAL SHRNA AND COMPOSITION INCLUDING THE SAME. Applicant: CUROCELL INC. KOREA ADVANCED INSTITUTE OF SCIENCE AND TECHNOLOGY. Application To Be Assigned. The sequence listing filed with the application follows.

SEQUENCE LISTING (290 sequences)

SEQ ID NO: 1 - DNA, 21 bp, Artificial Sequence
  partial shRNA sequence, included in shRNA to target GFP for RNA interference
tctcggcatggacgagctgta

SEQ ID NO: 2 - DNA, 21 bp, Artificial Sequence
  partial shRNA sequence, included in shRNA to target PD-1 for RNA interference
tggaacccattcctgaaatta

SEQ ID NO: 3 - DNA, 21 bp, Artificial Sequence
  partial shRNA sequence, included in shRNA to target PD-1 for RNA interference
ggaacccattcctgaaattat

SEQ ID NO: 4 - DNA, 21 bp, Artificial Sequence
  partial shRNA sequence, included in shRNA to target PD-1 for RNA interference
gaacccattcctgaaattatt

SEQ ID NO: 5 - DNA, 21 bp, Artificial Sequence
  partial shRNA sequence, included in shRNA to target PD-1 for RNA interference
acccattcctgaaattattta

SEQ ID NO: 6 - DNA, 21 bp, Artificial Sequence
  partial shRNA sequence, included in shRNA to target PD-1 for RNA interference
cccattcctgaaattatttaa

SEQ ID NO: 7 - DNA, 21 bp, Artificial Sequence
  partial shRNA sequence, included in shRNA to target PD-1 for RNA interference
ccttccctgtggttctattat

SEQ ID NO: 8 - DNA, 21 bp, Artificial Sequence
  partial shRNA sequence, included in shRNA to target PD-1 for RNA interference
cttccctgtggttctattata

SEQ ID NO: 9 - DNA, 21 bp, Artificial Sequence
  partial shRNA sequence, included in shRNA to target PD-1 for RNA interference
ttccctgtggttctattatat

SEQ ID NO: 10 - DNA, 21 bp, Artificial Sequence
  partial shRNA sequence, included in shRNA to target PD-1 for RNA interference
tccctgtggttctattatatt

SEQ ID NO: 11 - DNA, 21 bp, Artificial Sequence
  partial shRNA sequence, included in shRNA to target PD-1 for RNA interference
ccctgtggttctattatatta

SEQ ID NO: 12 - DNA, 21 bp, Artificial Sequence
  partial shRNA sequence, included in shRNA to target PD-1 for RNA interference
cctgtggttctattatattat

SEQ ID NO: 13 - DNA, 21 bp, Artificial Sequence
  partial shRNA sequence, included in shRNA to target TIM-3 for RNA interference
gatgaaagggatgtgaattat

SEQ ID NO: 14 - DNA, 21 bp, Artificial Sequence
  partial shRNA sequence, included in shRNA to target TIM-3 for RNA interference
gggagcctccctgatataaat

SEQ ID NO: 15 - DNA, 19 bp, Artificial Sequence
  partial shRNA sequence, included in shRNA to target TIM-3 for RNA interference
ggaattcgctcagaagaaa

SEQ ID NO: 16 - DNA, 21 bp, Artificial Sequence
  partial shRNA sequence, included in shRNA to target TIM-3 for RNA interference
ggaccaaactgaagctatatt

SEQ ID NO: 17 - DNA, 21 bp, Artificial Sequence
  partial shRNA sequence, included in shRNA to target TIM-3 for RNA interference
agaactttggtttcctttaat

SEQ ID NO: 18 - DNA, 21 bp, Artificial Sequence
  partial shRNA sequence, included in shRNA to target TIM-3 for RNA interference
atgaaagggatgtgaattatt

SEQ ID NO: 19 - DNA, 21 bp, Artificial Sequence
  partial shRNA sequence, included in shRNA to target TIM-3 for RNA interference
tcttatcttcggcgctttaat

SEQ ID NO: 20 - DNA, 21 bp, Artificial Sequence
  partial shRNA sequence, included in shRNA to target TIM-3 for RNA interference
cttatcttcggcgctttaatt

SEQ ID NO: 21 - DNA, 21 bp, Artificial Sequence
  partial shRNA sequence, included in shRNA to target TIM-3 for RNA interference
ttatcttcggcgctttaattt

SEQ ID NO: 22 - DNA, 21 bp, Artificial Sequence
  partial shRNA sequence, included in shRNA to target TIM-3 for RNA interference
gaggagcccaatgagtattat

SEQ ID NO: 23 - DNA, 21 bp, Artificial Sequence
  partial shRNA sequence, included in shRNA to target TIM-3 for RNA interference
aggagcccaatgagtattatt

SEQ ID NO: 24 - DNA, 21 bp, Artificial Sequence
  partial shRNA sequence, included in shRNA to target TIM-3 for RNA interference
atagatccaaccaccttattt

SEQ ID NO: 25 - DNA, 21 bp, Artificial Sequence
  partial shRNA sequence, included in shRNA to target TIM-3 for RNA interference
atgtcattgcctctgtattta

SEQ ID NO: 26 - DNA, 21 bp, Artificial Sequence
  partial shRNA sequence, included in shRNA to target TIM-3 for RNA interference
tgtcattgcctctgtatttaa

SEQ ID NO: 27 - DNA, 21 bp, Artificial Sequence
  partial shRNA sequence, included in shRNA to target TIM-3 for RNA interference
accaccatgcccagctaattt

SEQ ID NO: 28 - DNA, 21 bp, Artificial Sequence
  partial shRNA sequence, included in shRNA to target TIM-3 for RNA interference
tgttgagatttaggcttattt

SEQ ID NO: 29 - DNA, 21 bp, Artificial Sequence
  partial shRNA sequence, included in shRNA to target TIM-3 for RNA interference
gaccaaactgaagctatattt

SEQ ID NO: 30 - DNA, 21 bp, Artificial Sequence
  partial shRNA sequence, included in shRNA to target TIM-3 for RNA interference
aggccttcagcaatctatatt

SEQ ID NO: 31 - DNA, 21 bp, Artificial Sequence
  partial shRNA sequence, included in shRNA to target TIM-3 for RNA interference
ggccttcagcaatctatatta

SEQ ID NO: 32 - DNA, 21 bp, Artificial Sequence
  partial shRNA sequence, included in shRNA to target TIM-3 for RNA interference
gagtggtccctaaacttaaat

SEQ ID NO: 33 - DNA, 21 bp, Artificial Sequence
  partial shRNA sequence, included in shRNA to target TIM-3 for RNA interference
agtggtccctaaacttaaatt

SEQ ID NO: 34 - DNA, 21 bp, Artificial Sequence
  partial shRNA sequence, included in shRNA to target TIM-3 for RNA interference
gtggtccctaaacttaaattt

SEQ ID NO: 35 - DNA, 19 bp, Artificial Sequence
  partial shRNA sequence, included in shRNA to target TIM-3 for RNA interference
ctaacacaaatatccacat

SEQ ID NO: 36 - DNA, 21 bp, Artificial Sequence
  partial shRNA sequence, included in shRNA to target LAG-3 for RNA interference
tcagcagcccagtccaaataa

SEQ ID NO: 37 - DNA, 21 bp, Artificial Sequence
  partial shRNA sequence, included in shRNA to target LAG-3 for RNA interference
cagcagcccagtccaaataaa

SEQ ID NO: 38 - DNA, 21 bp, Artificial Sequence
  partial shRNA sequence, included in shRNA to target LAG-3 for RNA interference
tcaacgtctccatcatgtata

SEQ ID NO: 39 - DNA, 21 bp, Artificial Sequence
  partial shRNA sequence, included in shRNA to target LAG-3 for RNA interference
caacgtctccatcatgtataa

SEQ ID NO: 40 - DNA, 21 bp, Artificial Sequence
  partial shRNA sequence, included in shRNA to target LAG-3 for RNA interference
ctggagacaatggcgacttta

SEQ ID NO: 41 - DNA, 21 bp, Artificial Sequence
  partial shRNA sequence, included in shRNA to target LAG-3 for RNA interference
ctcagcagcccagtccaaata

SEQ ID NO: 42 - DNA, 21 bp, Artificial Sequence
  partial shRNA sequence, included in shRNA to target LAG-3 for RNA interference
agcagcccagtccaaataaac

SEQ ID NO: 43 - DNA, 21 bp, Artificial Sequence
  partial shRNA sequence, included in shRNA to target CTLA-4 for RNA interference
gggatcaaagctatctatata

SEQ ID NO: 44 - DNA, 21 bp, Artificial Sequence
  partial shRNA sequence, included in shRNA to target CTLA-4 for RNA interference
ggatcaaagctatctatataa

SEQ ID NO: 45 - DNA, 21 bp, Artificial Sequence
  partial shRNA sequence, included in shRNA to target CTLA-4 for RNA interference
ggcaacggaacccagatttat

SEQ ID NO: 46 - DNA, 21 bp, Artificial Sequence
  partial shRNA sequence, included in shRNA to target CTLA-4 for RNA interference
tgaagaagagagtccatattt

SEQ ID NO: 47 - DNA, 21 bp, Artificial Sequence
  partial shRNA sequence, included in shRNA to target CTLA-4 for RNA interference
ttggatgcggaacccaaatta

SEQ ID NO: 48 - DNA, 21 bp, Artificial Sequence
  partial shRNA sequence, included in shRNA to target CTLA-4 for RNA interference
agcatcacttgggattaatat

SEQ ID NO: 49 - DNA, 21 bp, Artificial Sequence
  partial shRNA sequence, included in shRNA to target CTLA-4 for RNA interference
tgatgtgggtcaaggaattaa

SEQ ID NO: 50 - DNA, 21 bp, Artificial Sequence
  partial shRNA sequence, included in shRNA to target CTLA-4 for RNA interference
agcgagggagaagactatatt

SEQ ID NO: 51 - DNA, 21 bp, Artificial Sequence
  partial shRNA sequence, included in shRNA to target CTLA-4 for RNA interference
tttacgtatgagacgtttata

SEQ ID NO: 52 - DNA, 21 bp, Artificial Sequence
  partial shRNA sequence, included in shRNA to target BTLA for RNA interference
gctcctgtatagtttacttcc

SEQ ID NO: 53 - DNA, 21 bp, Artificial Sequence
  partial shRNA sequence, included in shRNA to target BTLA for RNA interference
ggaaattaacctggttgatgc

SEQ ID NO: 54 - DNA, 21 bp, Artificial Sequence
  partial shRNA sequence, included in shRNA to target BTLA for RNA interference
gcaccaacagaatatgcatcc

SEQ ID NO: 55 - DNA, 21 bp, Artificial Sequence
  partial shRNA sequence, included in shRNA to target BTLA for RNA interference
gctcaacaggatgtcaaataa

SEQ ID NO: 56 - DNA, 21 bp, Artificial Sequence
  partial shRNA sequence, included in shRNA to target BTLA for RNA interference
gcatcttgctgttcttcttac

SEQ ID NO: 57 - DNA, 21 bp, Artificial Sequence
  partial shRNA sequence, included in shRNA to target BTLA for RNA interference
gcatttgtggacaacttatgt

SEQ ID NO: 58 - DNA, 21 bp, Artificial Sequence
  partial shRNA sequence, included in shRNA to target CD160 for RNA interference
ggaacgcgactaaacttaatc

SEQ ID NO: 59 - DNA, 21 bp, Artificial Sequence
  partial shRNA sequence, included in shRNA to target CD160 for RNA interference
gatgttcaccataagccaagt

SEQ ID NO: 60 - DNA, 21 bp, Artificial Sequence
  partial shRNA sequence, included in shRNA to target CD160 for RNA interference
gcaagatgagtctgactatgg

SEQ ID NO: 61 - DNA, 21 bp, Artificial Sequence
  partial shRNA sequence, included in shRNA to target CD160 for RNA interference
ggcacagagaagaatgcaaca

SEQ ID NO: 62 - DNA, 21 bp, Artificial Sequence
  partial shRNA sequence, included in shRNA to target CD160 for RNA interference
gggaagagatgctaaatatac

SEQ ID NO: 63 - DNA, 21 bp, Artificial Sequence
  partial shRNA sequence, included in shRNA to target CD160 for RNA interference
gcaaatcagtgtaatccttga

SEQ ID NO: 64 - DNA, 21 bp, Artificial Sequence
  partial shRNA sequence, included in shRNA to target VISTA for RNA interference
gcaacttctccatcaccatgc

SEQ ID NO: 65 - DNA, 21 bp, Artificial Sequence
  partial shRNA sequence, included in shRNA to target VISTA for RNA interference
gcaaagatgcaccatccaact

SEQ ID NO: 66 - DNA, 21 bp, Artificial Sequence
  partial shRNA sequence, included in shRNA to target VISTA for RNA interference
gcggatggacagcaacattca

SEQ ID NO: 67 - DNA, 21 bp, Artificial Sequence
  partial shRNA sequence, included in shRNA to target VISTA for RNA interference
ggacacttctgagtatgaagc

SEQ ID NO: 68 - DNA, 21 bp, Artificial Sequence
  partial shRNA sequence, included in shRNA to target VISTA for RNA interference
gggaaccacaatgcacgaaag

SEQ ID NO: 69 - DNA, 21 bp, Artificial Sequence
  partial shRNA sequence, included in shRNA to target VISTA for RNA interference
ggtgctttccaacacactttc

SEQ ID NO: 70 - DNA, 21 bp, Artificial Sequence
  partial shRNA sequence, included in shRNA to target TIGIT for RNA interference
gcttctggccatttgtaatgc

SEQ ID NO: 71 - DNA, 21 bp, Artificial Sequence
  partial shRNA sequence, included in shRNA to target TIGIT for RNA interference
gggagtacttctgcatctatc

SEQ ID NO: 72 - DNA, 21 bp, Artificial Sequence
  partial shRNA sequence, included in shRNA to target TIGIT for RNA interference
gctgcatgactacttcaatgt

SEQ ID NO: 73 - DNA, 21 bp, Artificial Sequence
  partial shRNA sequence, included in shRNA to target TIGIT for RNA interference
taacgtggatcttgatcataa

SEQ ID NO: 74 - DNA, 21 bp, Artificial Sequence
  partial shRNA sequence, included in shRNA to target TIGIT for RNA interference
ggagacatacacaggccttca

SEQ ID NO: 75 - DNA, 21 bp, Artificial Sequence
  partial shRNA sequence, included in shRNA to target TIGIT for RNA interference
gcatttgggccttgatctacc

SEQ ID NO: 76 - DNA, 21 bp, Artificial Sequence
  partial shRNA sequence, included in shRNA to target 2B4 for RNA interference
gacaggttgcaaggcagttct

SEQ ID NO: 77 - DNA, 21 bp, Artificial Sequence
  partial shRNA sequence, included in shRNA to target 2B4 for RNA interference
gggagtgcctcttcagttaca

SEQ ID NO: 78 - DNA, 21 bp, Artificial Sequence
  partial shRNA sequence, included in shRNA to target 2B4 for RNA interference
ggacgaggaggttgacattaa

SEQ ID NO: 79 - DNA, 21 bp, Artificial Sequence
  partial shRNA sequence, included in shRNA to target 2B4 for RNA interference
gaggagaaagaggaaggagaa

SEQ ID NO: 80 - DNA, 21 bp, Artificial Sequence
  partial shRNA sequence, included in shRNA to target 2B4 for RNA interference
gcccttccttcaatagcacta

SEQ ID NO: 81 - DNA, 21 bp, Artificial Sequence
  partial shRNA sequence, included in shRNA to target 2B4 for RNA interference
ggttgactgcatttctagact

SEQ ID NO: 82 - DNA, 21 bp, Artificial Sequence
  partial shRNA sequence, included in shRNA to target PD-L1 for RNA interference
gcatttgctgaacgcatttac

SEQ ID NO: 83 - DNA, 21 bp, Artificial Sequence
  partial shRNA sequence, included in shRNA to target PD-L1 for RNA interference
gctgcactaattgtctattgg

SEQ ID NO: 84 - DNA, 21 bp, Artificial Sequence
  partial shRNA sequence, included in shRNA to target PD-L1 for RNA interference
ggatccagtcacctctgaaca

SEQ ID NO: 85 - DNA, 21 bp, Artificial Sequence
  partial shRNA sequence, included in shRNA to target PD-L1 for RNA interference
gcacatcctccaaatgaaagg

SEQ ID NO: 86 - DNA, 21 bp, Artificial Sequence
  partial shRNA sequence, included in shRNA to target PD-L1 for RNA interference
ggattctcaacctgtggttta

SEQ ID NO: 87 - DNA, 21 bp, Artificial Sequence
  partial shRNA sequence, included in shRNA to target PD-L1 for RNA interference
ggtgcttggtctcctctataa

SEQ ID NO: 88 - DNA, 21 bp, Artificial Sequence
  partial shRNA sequence, included in shRNA to target CEACAM-1 for RNA interference
gcacagtactcctggcttatc

SEQ ID NO: 89 - DNA, 21 bp, Artificial Sequence
  partial shRNA sequence, included in shRNA to target CEACAM-1 for RNA interference
gcaacaggaccacagtcaaga

SEQ ID NO: 90 - DNA, 21 bp, Artificial Sequence
  partial shRNA sequence, included in shRNA to target CEACAM-1 for RNA interference
gcaacaccaccctcagcataa

SEQ ID NO: 91 - DNA, 21 bp, Artificial Sequence
  partial shRNA sequence, included in shRNA to target CEACAM-1 for RNA interference
gcctgttcagagcactcattc

SEQ ID NO: 92 - DNA, 21 bp, Artificial Sequence
  partial shRNA sequence, included in shRNA to target CEACAM-1 for RNA interference
gcagtaatgccttctcctatt

SEQ ID NO: 93 - DNA, 21 bp, Artificial Sequence
  partial shRNA sequence, included in shRNA to target CEACAM-1 for RNA interference
gcaccttggtgcttagctaga

SEQ ID NO: 94 - DNA, 21 bp, Artificial Sequence
  partial shRNA sequence, included in shRNA to target CEACAM-3 for RNA interference
gcttccatctatgaggaattg

SEQ ID NO: 95 - DNA, 21 bp, Artificial Sequence
  partial shRNA sequence, included in shRNA to target CEACAM-3 for RNA interference
gccagagaaccagctataagt

SEQ ID NO: 96 - DNA, 21 bp, Artificial Sequence
  partial shRNA sequence, included in shRNA to target CEACAM-3 for RNA interference
gggtccctgatgaatatctgg

SEQ ID NO: 97 - DNA, 21 bp, Artificial Sequence
  partial shRNA sequence, included in shRNA to target CEACAM-3 for RNA interference
ggcttgcagggaaagtgaatg

SEQ ID NO: 98 - DNA, 21 bp, Artificial Sequence
  partial shRNA sequence, included in shRNA to target CEACAM-3 for RNA interference
gcttgcagggaaagtgaatgg

SEQ ID NO: 99 - DNA, 21 bp, Artificial Sequence
  partial shRNA sequence, included in shRNA to target CEACAM-3 for RNA interference
agcttccatctatgaggaatt

SEQ ID NO: 100 - DNA, 21 bp, Artificial Sequence
  partial shRNA sequence, included in shRNA to target CEACAM-5 for RNA interference
ggaatccagaacgaattaagt

SEQ ID NO: 101 - DNA, 21 bp, Artificial Sequence
  partial shRNA sequence, included in shRNA to target CEACAM-5 for RNA interference
ggctgattgatgggaacatcc

SEQ ID NO: 102 - DNA, 21 bp, Artificial Sequence
  partial shRNA sequence, included in shRNA to target CEACAM-5 for RNA interference
ggactacagtcaagacaatca

SEQ ID NO: 103 - DNA, 21 bp, Artificial Sequence
  partial shRNA sequence, included in shRNA to target CEACAM-5 for RNA interference
ggaccctcactctattcaatg

SEQ ID NO: 104 - DNA, 21 bp, Artificial Sequence
  partial shRNA sequence, included in shRNA to target CEACAM-5 for RNA interference
gctactggccgcaataattcc

SEQ ID NO: 105 - DNA, 21 bp, Artificial Sequence
  partial shRNA sequence, included in shRNA to target CEACAM-5 for RNA interference
gctctttgtatgacagaatac

SEQ ID NO: 106 - DNA, 21 bp, Artificial Sequence
  partial shRNA sequence, included in shRNA to target CD96 for RNA interference
ggtccaaggtcaccaataaga

SEQ ID NO: 107 - DNA, 21 bp, Artificial Sequence
  partial shRNA sequence, included in shRNA to target CD96 for RNA interference
gcaaccatacgatagaaatag

SEQ ID NO: 108 - DNA, 21 bp, Artificial Sequence
  partial shRNA sequence, included in shRNA to target CD96 for RNA interference
ggttctgaaatttcctcaaca

SEQ ID NO: 109 - DNA, 21 bp, Artificial Sequence
  partial shRNA sequence, included in shRNA to target CD96 for RNA interference
gcaagatatccagctacatct

SEQ ID NO: 110 - DNA, 21 bp, Artificial Sequence
  partial shRNA sequence, included in shRNA to target CD96 for RNA interference
gcaactcaccctcttccatct

SEQ ID NO: 111 - DNA, 21 bp, Artificial Sequence
  partial shRNA sequence, included in shRNA to target CD96 for RNA interference
gctgcattccctaagataatt

SEQ ID NO: 112 - DNA, 21 bp, Artificial Sequence
  partial shRNA sequence, included in shRNA to target LAIR1 for RNA interference
gggacagtagatccacataca

SEQ ID NO: 113 - DNA, 21 bp, Artificial Sequence
  partial shRNA sequence, included in shRNA to target LAIR1 for RNA interference
ggacaacagtcacaatgagca

SEQ ID NO: 114 - DNA, 21 bp, Artificial Sequence
  partial shRNA sequence, included in shRNA to target LAIR1 for RNA interference
ggctgttgatgttctagagag

SEQ ID NO: 115 - DNA, 21 bp, Artificial Sequence
  partial shRNA sequence, included in shRNA to target LAIR1 for RNA interference
gcagacaaggccacagtcaat

SEQ ID NO: 116 - DNA, 21 bp, Artificial Sequence
  partial shRNA sequence, included in shRNA to target LAIR1 for RNA interference
ggaggtttctaaccagcatcc

SEQ ID NO: 117 - DNA, 21 bp, Artificial Sequence
  partial shRNA sequence, included in shRNA to target LAIR1 for RNA interference
gccttgagactgtgctataca

SEQ ID NO: 118 - DNA, 21 bp, Artificial Sequence
  partial shRNA sequence, included in shRNA to target KLRG1 for RNA interference
ccaagcccagaatgactatgg

SEQ ID NO: 119 - DNA, 21 bp, Artificial Sequence
  partial shRNA sequence, included in shRNA to target KLRG1 for RNA interference
gccttcttgttcttgccttgt

SEQ ID NO: 120 - DNA, 21 bp, Artificial Sequence
  partial shRNA sequence, included in shRNA to target KLRG1 for RNA interference
gcttctgactgcagttcttct

SEQ ID NO: 121 - DNA, 21 bp, Artificial Sequence
  partial shRNA sequence, included in shRNA to target KLRG1 for RNA interference
gctggatgaaatatggtaacc

SEQ ID NO: 122 - DNA, 21 bp, Artificial Sequence
  partial shRNA sequence, included in shRNA to target KLRG1 for RNA interference
ggaaatgagcctgctccaagt

SEQ ID NO: 123 - DNA, 21 bp, Artificial Sequence
  partial shRNA sequence, included in shRNA to target KLRG1 for RNA interference
ggattggtctgaggaacaatt

SEQ ID NO: 124 - DNA, 21 bp, Artificial Sequence
  partial shRNA sequence, included in shRNA to target FAS for RNA interference
gccaagaagggaaggagtaca

SEQ ID NO: 125 - DNA, 21 bp, Artificial Sequence
  partial shRNA sequence, included in shRNA to target FAS for RNA interference
gccaattccactaattgtttg

SEQ ID NO: 126 - DNA, 21 bp, Artificial Sequence
  partial shRNA sequence, included in shRNA to target FAS for RNA interference
ggttctcatgaatctccaact

SEQ ID NO: 127 - DNA, 21 bp, Artificial Sequence
  partial shRNA sequence, included in shRNA to target FAS for RNA interference
gctggagtcatgacactaagt

SEQ ID NO: 128 - DNA, 21 bp, Artificial Sequence
  partial shRNA sequence, included in shRNA to target FAS for RNA interference
gcctggtttggagatactaac

SEQ ID NO: 129 - DNA, 21 bp, Artificial Sequence
  partial shRNA sequence, included in shRNA to target FAS for RNA interference
ggaaccacctaaagaacttcc

SEQ ID NO: 130 - DNA, 21 bp, Artificial Sequence
  partial shRNA sequence, included in shRNA to target Cbl-b for RNA interference
ccgcgttgatttaaagaaaga

SEQ ID NO: 131 - DNA, 21 bp, Artificial Sequence
  partial shRNA sequence, included in shRNA to target Cbl-b for RNA interference
gcctgatacatatcagcattt

SEQ ID NO: 132 - DNA, 21 bp, Artificial Sequence
  partial shRNA sequence, included in shRNA to target Cbl-b for RNA interference
gcggaattggaatttcttagc

SEQ ID NO: 133 - DNA, 21 bp, Artificial Sequence
  partial shRNA sequence, included in shRNA to target Cbl-b for RNA interference
gcacgactacagaaatatagc

SEQ ID NO: 134 - DNA, 21 bp, Artificial Sequence
  partial shRNA sequence, included in shRNA to target Cbl-b for RNA interference
tttccggttaagttgcactcg

SEQ ID NO: 135 - DNA, 21 bp, Artificial Sequence
  partial shRNA sequence, included in shRNA to target Cbl-b for RNA interference
gcctggatctaattcagaaag

SEQ ID NO: 136 - DNA, 21 bp, Artificial Sequence
  partial shRNA sequence, included in shRNA to target LRR1 for RNA interference
gaaagccactgttcggttaaa

SEQ ID NO: 137 - DNA, 21 bp, Artificial Sequence
  partial shRNA sequence, included in shRNA to target LRR1 for RNA interference
tcctgtggatatctgtctaag

SEQ ID NO: 138 - DNA, 21 bp, Artificial Sequence
  partial shRNA sequence, included in shRNA to target LRR1 for RNA interference
ggctcatagaggctgtaatgt

SEQ ID NO: 139 - DNA, 21 bp, Artificial Sequence
  partial shRNA sequence, included in shRNA to target LRR1 for RNA interference
gggcttgtccgagttgatatg

SEQ ID NO: 140 - DNA, 21 bp, Artificial Sequence
  partial shRNA sequence, included in shRNA to target LRR1 for RNA interference
aagatttggataccgcaaaaa

SEQ ID NO: 141 - DNA, 21 bp, Artificial Sequence
  partial shRNA sequence, included in shRNA to target LRR1 for RNA interference
gtggtactgaagcacctatta

SEQ ID NO: 142 - DNA, 21 bp, Artificial Sequence
  partial shRNA sequence, included in shRNA to target TGFBR1 for RNA interference
gcttgttcagagaacaattgc

SEQ ID NO: 143 - DNA, 21 bp, Artificial Sequence
  partial shRNA sequence, included in shRNA to target TGFBR1 for RNA interference
ggagattgttggtacccaagg

SEQ ID NO: 144 - DNA, 21 bp, Artificial Sequence
  partial shRNA sequence, included in shRNA to target TGFBR1 for RNA interference
gcagctaggcttacagcattg

SEQ ID NO: 145 - DNA, 21 bp, Artificial Sequence
  partial shRNA sequence, included in shRNA to target TGFBR1 for RNA interference
ggtcctttctgtgcactatga

SEQ ID NO: 146 - DNA, 21 bp, Artificial Sequence
  partial shRNA sequence, included in shRNA to target TGFBR1 for RNA interference
ggtggtagctaaagaacattc

SEQ ID NO: 147 - DNA, 21 bp, Artificial Sequence
  partial shRNA sequence, included in shRNA to target TGFBR1 for RNA interference
ggacctgtctacaggtgatct

SEQ ID NO: 148 - DNA, 21 bp, Artificial Sequence
  partial shRNA sequence, included in shRNA to target DNMT3A for RNA interference
gccaaggtcattgcaggaatg

SEQ ID NO: 149 - DNA, 21 bp, Artificial Sequence
  partial shRNA sequence, included in shRNA to target DNMT3A for RNA interference
gcagaacaagcccatgattga

SEQ ID NO: 150 - DNA, 21 bp, Artificial Sequence
  partial shRNA sequence, included in shRNA to target DNMT3A for RNA interference
cccaaggtcaaggagattatt

SEQ ID NO: 151 - DNA, 21 bp, Artificial Sequence
  partial shRNA sequence, included in shRNA to target DNMT3A for RNA interference
gcagaagtgccggaacattga

SEQ ID NO: 152 - DNA, 21 bp, Artificial Sequence
  partial shRNA sequence, included in shRNA to target DNMT3A for RNA interference
gcgtcacacagaagcatatcc

SEQ ID NO: 153 - DNA, 21 bp, Artificial Sequence
  partial shRNA sequence, included in shRNA to target DNMT3A for RNA interference
ccggctcttctttgagttcta

SEQ ID NO: 154 - DNA, 21 bp, Artificial Sequence
  partial shRNA sequence, included in shRNA to target A2aR for RNA interference
cagaacgtcaccaactacttt

SEQ ID NO: 155 - DNA, 21 bp, Artificial Sequence
  partial shRNA sequence, included in shRNA to target A2aR for RNA interference
ccatgctaggttggaacaact

SEQ ID NO: 156 - DNA, 21 bp, Artificial Sequence
  partial shRNA sequence, included in shRNA to target A2aR for RNA interference
ccaagtggcctgtctctttga

SEQ ID NO: 157 - DNA, 21 bp, Artificial Sequence
  partial shRNA sequence, included in shRNA to target A2aR for RNA interference
ggtgtctatttgcggatcttc

SEQ ID NO: 158 - DNA, 21 bp, Artificial Sequence
  partial shRNA sequence, included in shRNA to target A2aR for RNA interference
agaccttccgcaagatcattc

SEQ ID NO: 159 - DNA, 21 bp, Artificial Sequence
  partial shRNA sequence, included in shRNA to target A2aR for RNA interference
tccttagccatgagctcaagg

SEQ ID NO: 160 - DNA, 21 bp, Artificial Sequence
  partial shRNA sequence, included in shRNA to target Cbl-c for RNA interference
gaaagtactgtggacacatgt

SEQ ID NO: 161 - DNA, 21 bp, Artificial Sequence
  partial shRNA sequence, included in shRNA to target Cbl-c for RNA interference
gcacgtgtccatcttcgagtt

SEQ ID NO: 162 - DNA, 21 bp, Artificial Sequence
  partial shRNA sequence, included in shRNA to target Cbl-c for RNA interference
ggccaacactcctcaagaact

SEQ ID NO: 163 - DNA, 21 bp, Artificial Sequence
  partial shRNA sequence, included in shRNA to target Cbl-c for RNA interference
ggcttctacctctacccagat

SEQ ID NO: 164 - DNA, 21 bp, Artificial Sequence
  partial shRNA sequence, included in shRNA to target Cbl-c for RNA interference
ggccatggactccacatttga

SEQ ID NO: 165 - DNA, 21 bp, Artificial Sequence
  partial shRNA sequence, included in shRNA to target Cbl-c for RNA interference
ggccgtgagtatctaccagtt

SEQ ID NO: 166 - DNA, 21 bp, Artificial Sequence
  partial shRNA sequence, included in shRNA to target DGK alpha for RNA interference
gccagaagacaagttagaatt

SEQ ID NO: 167 - DNA, 21 bp, Artificial Sequence
  partial shRNA sequence, included in shRNA to target DGK alpha for RNA interference
gctctggaagttccagtatat

SEQ ID NO: 168 - DNA, 21 bp, Artificial Sequence
  partial shRNA sequence, included in shRNA to target DGK alpha for RNA interference
ggaaatgatctggctcgatgc

SEQ ID NO: 169 - DNA, 21 bp, Artificial Sequence
  partial shRNA sequence, included in shRNA to target DGK alpha for RNA interference
gcaaagatcctcaaggattta

SEQ ID NO: 170 - DNA, 21 bp, Artificial Sequence
  partial shRNA sequence, included in shRNA to target DGK alpha for RNA interference
ggatgcctctattgctcatcg

SEQ ID NO: 171 - DNA, 21 bp, Artificial Sequence
  partial shRNA sequence, included in shRNA to target DGK alpha for RNA interference
gctatggtacttcgaatttgc

SEQ ID NO: 172 - DNA, 21 bp, Artificial Sequence
  partial shRNA sequence, included in shRNA to target DGK zeta for RNA interference
ggaagggattccagcagaagt

SEQ ID NO: 173 - DNA, 21 bp, Artificial Sequence
  partial shRNA sequence, included in shRNA to target DGK zeta for RNA interference
gcaaggagattgtggccatca

SEQ ID NO: 174 - DNA, 21 bp, Artificial Sequence
  partial shRNA sequence, included in shRNA to target DGK zeta for RNA interference
gggcatccttcaagaggaagt

SEQ ID NO: 175 - DNA, 21 bp, Artificial Sequence
  partial shRNA sequence, included in shRNA to target DGK zeta for RNA interference
gcaaagatcatccagtctttc

SEQ ID NO: 176 - DNA, 21 bp, Artificial Sequence
  partial shRNA sequence, included in shRNA to target DGK zeta for RNA interference
gctggagatgtaccgcaaagt

SEQ ID NO: 177 - DNA, 21 bp, Artificial Sequence
  partial shRNA sequence, included in shRNA to target DGK zeta for RNA interference
gcacaggatgagatttatatc

SEQ ID NO: 178 - DNA, 21 bp, Artificial Sequence
  partial shRNA sequence, included in shRNA to target MerTK for RNA interference
ggaagaccacatacaggaaac

SEQ ID NO: 179 - DNA, 21 bp, Artificial Sequence
  partial shRNA sequence, included in shRNA to target MerTK for RNA interference
gcattggtgtttcctgcatga

SEQ ID NO: 180 - DNA, 21 bp, Artificial Sequence
  partial shRNA sequence, included in shRNA to target MerTK for RNA interference
gcacacggttgggtagattat

SEQ ID NO: 181 - DNA, 21 bp, Artificial Sequence
  partial shRNA sequence, included in shRNA to target MerTK for RNA interference
gggtctgtaatggaaggaaat

SEQ ID NO: 182 - DNA, 21 bp, Artificial Sequence
  partial shRNA sequence, included in shRNA to target MerTK for RNA interference
gcatgttgcgagatgacatga

SEQ ID NO: 183 - DNA, 21 bp, Artificial Sequence
  partial shRNA sequence, included in shRNA to target MerTK for RNA interference
gcagaccgagtctacacaagt

SEQ ID NO: 184 - DNA, 21 bp, Artificial Sequence
  partial shRNA sequence, included in shRNA to target SHP1 for RNA interference
gcaccatcatccacctcaagt

SEQ ID NO: 185 - DNA, 21 bp, Artificial Sequence
  partial shRNA sequence, included in shRNA to target SHP1 for RNA interference
ggtcacccacatcaaggtcat

SEQ ID NO: 186 - DNA, 21 bp, Artificial Sequence
  partial shRNA sequence, included in shRNA to target SHP1 for RNA interference
gggcaagaaccgctacaagaa

SEQ ID NO: 187 - DNA, 21 bp, Artificial Sequence
  partial shRNA sequence, included in shRNA to target SHP1 for RNA interference
ggaacaaatgcgtcccatact

SEQ ID NO: 188 - DNA, 21 bp, Artificial Sequence
  partial shRNA sequence, included in shRNA to target SHP1 for RNA interference
gcctggactgtgacattgaca

SEQ ID NO: 189 - DNA, 21 bp, Artificial Sequence
  partial shRNA sequence, included in shRNA to target SHP1 for RNA interference
gaacctgcacactaagaacaa

SEQ ID NO: 190 - DNA, 21 bp, Artificial Sequence
  partial shRNA sequence, included in shRNA to target SHP2 for RNA interference
gcagatcctacctctgaaagg

SEQ ID NO: 191 - DNA, 21 bp, Artificial Sequence
  partial shRNA sequence, included in shRNA to target SHP2 for RNA interference
gcaatgacggcaagtctaaag

SEQ ID NO: 192 - DNA, 21 bp, Artificial Sequence
  partial shRNA sequence, included in shRNA to target SHP2 for RNA interference
ggaactgaaatacgacgttgg

SEQ ID NO: 193 - DNA, 21 bp, Artificial Sequence
  partial shRNA sequence, included in shRNA to target SHP2 for RNA interference
gcgtgttaggaacgtcaaaga

SEQ ID NO: 194 - DNA, 21 bp, Artificial Sequence
  partial shRNA sequence, included in shRNA to target SHP2 for RNA interference
gctcatgactatacgctaaga

SEQ ID NO: 195 - DNA, 21 bp, Artificial Sequence
  partial shRNA sequence, included in shRNA to target SHP2 for RNA interference
ggagagaacggtctggcaata

SEQ ID NO: 196 - DNA, 21 bp, Artificial Sequence
  partial shRNA sequence, included in shRNA to target PP2A for RNA interference
gcagctgaacgagaaccaagt

SEQ ID NO: 197 - DNA, 21 bp, Artificial Sequence
  partial shRNA sequence, included in shRNA to target PP2A for RNA interference
ggagactgtgactcttcttgt

SEQ ID NO: 198 - DNA, 21 bp, Artificial Sequence
  partial shRNA sequence, included in shRNA to target PP2A for RNA interference
ggaatgccaacgtttggaaat

SEQ ID NO: 199 - DNA, 21 bp, Artificial Sequence
  partial shRNA sequence, included in shRNA to target PP2A for RNA interference
ggatcgtttacaggaagttcc

SEQ ID NO: 200 - DNA, 21 bp, Artificial Sequence
  partial shRNA sequence, included in shRNA to target PP2A for RNA interference
gcctttgtatgtggaagtata

SEQ ID NO: 201 - DNA, 21 bp, Artificial Sequence
  partial shRNA sequence, included in shRNA to target PP2A for RNA interference
gcctgctgtatttatagtaac

SEQ ID NO: 202 - DNA, 21 bp, Artificial Sequence
  partial shRNA sequence, included in shRNA to target CD45 for RNA interference
gctgcacatcaaggagtaatt

SEQ ID NO: 203 - DNA, 21 bp, Artificial Sequence
  partial shRNA sequence, included in shRNA to target CD45 for RNA interference
gctggaaatactctggttaga

SEQ ID NO: 204 - DNA, 21 bp, Artificial Sequence
  partial shRNA sequence, included in shRNA to target CD45 for RNA interference
ggagcttgttgaaagggatga

SEQ ID NO: 205 - DNA, 21 bp, Artificial Sequence
  partial shRNA sequence, included in shRNA to target CD45 for RNA interference
gcagaatactggccgtcaatg

SEQ ID NO: 206 - DNA, 21 bp, Artificial Sequence
  partial shRNA sequence, included in shRNA to target CD45 for RNA interference
ggttatgttgtcaagctaagg

SEQ ID NO: 207 - DNA, 21 bp, Artificial Sequence
  partial shRNA sequence, included in shRNA to target CD45 for RNA interference
gcagaacccaaggaattaatc

SEQ ID NO: 208 - DNA, 21 bp, Artificial Sequence
  partial shRNA sequence, included in shRNA to target CD148 for RNA interference
ggtgtaacatcacaggcttac

SEQ ID NO: 209 - DNA, 21 bp, Artificial Sequence
  partial shRNA sequence, included in shRNA to target CD148 for RNA interference
gccatagagttcaggacaaat

SEQ ID NO: 210 - DNA, 21 bp, Artificial Sequence
  partial shRNA sequence, included in shRNA to target CD148 for RNA interference
gcaattctcgggtagaaataa

SEQ ID NO: 211 - DNA, 21 bp, Artificial Sequence
  partial shRNA sequence, included in shRNA to target CD148 for RNA interference
gctggcttcaccaacattacc

SEQ ID NO: 212 - DNA, 21 bp, Artificial Sequence
  partial shRNA sequence, included in shRNA to target CD148 for RNA interference
gggagcaaatcatctgcattc

SEQ ID NO: 213 - DNA, 21 bp, Artificial Sequence
  partial shRNA sequence, included in shRNA to target CD148 for RNA interference
gcgactcaaatatcaccttga

SEQ ID NO: 214 - DNA, 21 bp, Artificial Sequence
  partial shRNA sequence, included in shRNA to target IL-10R alpha for RNA interference
gctcctgaggtatggaataga

SEQ ID NO: 215 - DNA, 21 bp, Artificial Sequence
  partial shRNA sequence, included in shRNA to target IL-10R alpha for RNA interference
gcaaatgacacatatgaaagc

SEQ ID NO: 216 - DNA, 21 bp, Artificial Sequence
  partial shRNA sequence, included in shRNA to target IL-10R alpha for RNA interference
ggtctaaagaggagtgcatct

SEQ ID NO: 217 - DNA, 21 bp, Artificial Sequence
  partial shRNA sequence, included in shRNA to target IL-10R alpha for RNA interference
gggctatttgaaacaggatcc

SEQ ID NO: 218 - DNA, 21 bp, Artificial Sequence
  partial shRNA sequence, included in shRNA to target IL-10R alpha for RNA interference
gctgtaggaatggaagcttca

SEQ ID NO: 219 - DNA, 21 bp, Artificial Sequence
  partial shRNA sequence, included in shRNA to target IL-10R alpha for RNA interference
gcttgtgtttgctgctaatgt

SEQ ID NO: 220 - DNA, 726 bp, Artificial Sequence
  mU6-shTIM-3-><-shPD-1-hU6
gttaacaaggtcgggcaggaagagggcctatttcccatgattccttcatatttgcatatacgatacaaggctgttagagagataattagaattaatttgactgtaaacacaaagatattagtacaaaatacgtgacgtagaaagtaataatttcttgggtagtttgcagttttaaaattatgttttaaaatggactatcatatgcttaccgtaacttgaaagtatttcgatttcttggctttatatatcttgtggaaaggacgaaacaccgcctgtggttctattatattatttcaagagaataatataatagaaccacaggtttttgactagtcaaaaaggaattcgctcagaagaaatctcttgaatttcttctgagcgaattccaaacaaggcttttctccaagggatatttatagtctcaaaacacacaattactttacagttagggtgagtttccttttgtgctgttttttaaaataataatttagtatttgtatctcttatagaaatccaagcctatcatgtaaaatgtagctagtattaaaaagaacagattatctgtcttttatcgcacattaagcctctatagttactaggaaatattatatgcaaattaaccggggcaggggagtagccgagcttctcccacaagtctgtgcgagggggccggcgcgggcctagagatggcggcgtcggatcgctagccatatgtctagagtatac

SEQ ID NO: 221 - DNA, 726 bp, Artificial Sequence
  shTIM-3-mU6<-->hU6-shPD-1
gttaaccaaaaacctgtggttctattatattattctcttgaaataatataatagaaccacaggcggtgtttcgtcctttccacaagatatataaagccaagaaatcgaaatactttcaagttacggtaagcatatgatagtccattttaaaacataattttaaaactgcaaactacccaagaaattattactttctacgtcacgtattttgtactaatatctttgtgtttacagtcaaattaattctaattatctctctaacagccttgtatcgtatatgcaaatatgaaggaatcatgggaaataggccctcttcctgcccgaccttactagtgatccgacgccgccatctctaggcccgcgccggccccctcgcacagacttgtgggagaagctcggctactcccctgccccggttaatttgcatataatatttcctagtaactatagaggcttaatgtgcgataaaagacagataatctgttctttttaatactagctacattttacatgataggcttggatttctataagagatacaaatactaaattattattttaaaaaacagcacaaaaggaaactcaccctaactgtaaagtaattgtgtgttttgagactataaatatcccttggagaaaagccttgtttggaattcgctcagaagaaattcaagagatttcttctgagcgaattcctttttggctagccatatgtctagagtatac

SEQ ID NO: 222 - DNA, 385 bp, Artificial Sequence
  shRNA cassette base sequence
  misc_feature (323)..(343): n is a, c, g, or t
  misc_feature (353)..(373): n is a, c, g, or t
gttaacgatccgacgccgccatctctaggcccgcgccggccccctcgcacagacttgtgggagaagctcggctactcccctgccccggttaatttgcatataatatttcctagtaactatagaggcttaatgtgcgataaaagacagataatctgttctttttaatactagctacattttacatgataggcttggatttctataagagatacaaatactaaattattattttaaaaaacagcacaaaaggaaactcaccctaactgtaaagtaattgtgtgttttgagactataaatatcccttggagaaaagccttgtttgnnnnnnnnnnnnnnnnnnnnnttcaagagannnnnnnnnnnnnnnnnnnnntttttggttaac

SEQ ID NO: 223 - DNA, 409 bp, Artificial Sequence
  mU6-shPD-1 MCS base sequence
gttaacgatccgacgccgccatctctaggcccgcgccggccccctcgcacagacttgtgggagaagctcggctactcccctgccccggttaatttgcatataatatttcctagtaactatagaggcttaatgtgcgataaaagacagataatctgttctttttaatactagctacattttacatgataggcttggatttctataagagatacaaatactaaattattattttaaaaaacagcacaaaaggaaactcaccctaactgtaaagtaattgtgtgttttgagactataaatatcccttggagaaaagccttgtttgcctgtggttctattatattatttcaagagaataatataatagaaccacaggtttttgactagtgctagccatatgtctagagtatac

SEQ ID NO: 224 - DNA, 328 bp, Artificial Sequence
  hU6-shPD-1 base sequence
gttaacaaggtcgggcaggaagagggcctatttcccatgattccttcatatttgcatatacgatacaaggctgttagagagataattagaattaatttgactgtaaacacaaagatattagtacaaaatacgtgacgtagaaagtaataatttcttgggtagtttgcagttttaaaattatgttttaaaatggactatcatatgcttaccgtaacttgaaagtatttcgatttcttggctttatatatcttgtggaaaggacgaaacaccgcctgtggttctattatattatttcaagagaataatataatagaaccacaggtttttg

SEQ ID NO: 225 - protein, 468 aa, Artificial Sequence
  CD22-CAR
QVQLQQSGPGLVKPSQTLSLTCAISGDSVSSNSAAWNWIRQSPSRGLEWLGRTYYRSKWYNDYAVSVKSRITINPDTSKNQFSLQLNSVTPEDTAVYYCAREVTGDLEDAFDIWGQGTMVTVSSGGGGSGGGGSGGGGSDIQMTQSPSSLSASVGDRVTITCRASQTIWSYLNWYQQRPGKAPNLLIYAASSLQSGVPSRFSGRGSGTDFTLTISSLQAEDFATYYCQQSYSIPQTFGQGTKLEITTTPAPRPPTPAPTIASQPLSLRPEACRPAAGGAVHTRGLDFACDIYIWAPLAGTCGVLLLSLVITLYCKRGRKKLLYIFKQPFMRPVQTTQEEDGCSCRFPEEEEGGCELRVKFSRSADAPAYKQGQNQLYNELNLGRREEYDVLDKRRGRDPEMGGKPRRKNPQEGLYNELQKDKMAEAYSEIGMKGERRRGKGHDGLYQGLSTATKDTYDALHMQALPPR

SEQ ID NO: 226 - protein, 486 aa, Artificial Sequence
  CD19-CAR
MALPVTALLLPLALLLHAARPDIQMTQTTSSLSASLGDRVTISCRASQDISKYLNWYQQKPDGTVKLLIYHTSRLHSGVPSRFSGSGSGTDYSLTISNLEQEDIATYFCQQGNTLPYTFGGGTKLEITGGGGSGGGGSGGGGSEVKLQESGPGLVAPSQSLSVTCTVSGVSLPDYGVSWIRQPPRKGLEWLGVIWGSETTYYNSALKSRLTIIKDNSKSQVFLKMNSLQTDDTAIYYCAKHYYYGGSYAMDYWGQGTSVTVSSTTTPAPRPPTPAPTIASQPLSLRPEACRPAAGGAVHTRGLDFACDIYIWAPLAGTCGVLLLSLVITLYCKRGRKKLLYIFKQPFMRPVQTTQEEDGCSCRFPEEEEGGCELRVKFSRSADAPAYKQGQNQLYNELNLGRREEYDVLDKRRGRDPEMGGKPRRKNPQEGLYNELQKDKMAEAYSEIGMKGERRRGKGHDGLYQGLSTATKDTYDALHMQALPPR

SEQ ID NO: 227 - protein, 782 aa, Artificial Sequence
  Delta LNGFR_P2A_CD19-CAR
MGAGATGRAMDGPRLLLLLLLGVSLGGAKEACPTGLYTHSGECCKACNLGEGVAQPCGANQTVCEPCLDSVTFSDVVSATEPCKPCTECVGLQSMSAPCVEADDAVCRCAYGYYQDETTGRCEACRVCEAGSGLVFSCQDKQNTVCEECPDGTYSDEANHVDPCLPCTVCEDTERQLRECTRWADAECEEIPGRWITRSTPPEGSDSTAPSTQEPEAPPEQDLIASTVAGVVTTVMGSSQPVVTRGTTDNLIPVYCSILAAVVVGLVAYIAFKRWGSGATNFSLLKQAGDVEENPGPALPVTALLLPLALLLHAARPDIQMTQTTSSLSASLGDRVTISCRASQDISKYLNWYQQKPDGTVKLLIYHTSRLHSGVPSRFSGSGSGTDYSLTISNLEQEDIATYFCQQGNTLPYTFGGGTKLEITGGGGSGGGGSGGGGSEVKLQESGPGLVAPSQSLSVTCTVSGVSLPDYGVSWIRQPPRKGLEWLGVIWGSETTYYNSALKSRLTIIKDNSKSQVFLKMNSLQTDDTAIYYCAKHYYYGGSYAMDYWGQGTSVTVSSTTTPAPRPPTPAPTIASQPLSLRPEACRPAAGGAVHTRGLDFACDIYIWAPLAGTCGVLLLSLVITLYCKRGRKKLLYIFKQPFMRPVQTTQEEDGCSCRFPEEEEGGCELRVKFSRSADAPAYKQGQNQLYNELNLGRREEYDVLDKRRGRDPEMGGKPRRKNPQEGLYNELQKDKMAEAYSEIGMKGERRRGKGHDGLYQGLSTATKDTYDALHMQALPPR

SEQ ID NO: 228 - DNA, 47 bp, Artificial Sequence
  Forward PCR cloning primer #1
ggtatactctagacatatggctagcactagtcaaaaacctgtggttc

SEQ ID NO: 229 - DNA, 26 bp, Artificial Sequence
  Reverse PCR cloning primer #1
ttgtaccgttaacgatccgacgccgc

SEQ ID NO: 230 - DNA, 102 bp, Artificial Sequence
  Forward PCR cloning primer #2
tgactagtcaaaaacctgtggttctattatattattctcttgaaataatataatagaaccacaggcggtgtttcgtcctttccacaagatatataaagccaa

SEQ ID NO: 231 - DNA, 50 bp, Artificial Sequence
  Reverse PCR cloning primer #2
gtaccgttaacaaggtcgggcaggaagagggcctatttcccatgattcct

SEQ ID NO: 232 - DNA, 39 bp, Artificial Sequence
  Forward PCR cloning primer #3
aggactagtcaaaaaggaattcgctcagaagaaatctct

SEQ ID NO: 233 - DNA, 27 bp, Artificial Sequence
  Reverse PCR cloning primer #3
ctagctagcgatccgacgccgccatct

SEQ ID NO: 234 - DNA, 42 bp, Artificial Sequence
  Forward PCR cloning primer #4
atgttaaccaaaaacctgtggttctattatattattctcttg

SEQ ID NO: 235 - DNA, 34 bp, Artificial Sequence
  Reverse PCR cloning primer #4
tcactagtaaggtcgggcaggaagagggcctatt

SEQ ID NO: 236 - DNA, 29 bp, Artificial Sequence
  Forward PCR cloning primer #5
taggccctcactagtgatccgacgccgcc

SEQ ID NO: 237 - DNA, 38 bp, Artificial Sequence
  Reverse PCR cloning primer #5
ctagctagccaaaaaggaattcgctcagaagaaatctc

SEQ ID NO: 238 - DNA, 21 bp, Artificial Sequence
  TIGIT-268
gcttctggccatttgtaatgc

SEQ ID NO: 239 - DNA, 21 bp, Artificial Sequence
  TIGIT-2
gggagtacttctgcatctatc

SEQ ID NO: 240 - DNA, 21 bp, Artificial Sequence
  TIGIT-739
gctgcatgactacttcaatgt

SEQ ID NO: 241 - DNA, 21 bp, Artificial Sequence
  TIGIT-1
taacgtggatcttgatcataa

SEQ ID NO: 242 - DNA, 21 bp, Artificial Sequence
  TIGIT-1386
ggagacatacacaggccttca

SEQ ID NO: 243 - DNA, 21 bp, Artificial Sequence
  TIGIT-1750
gcatttgggccttgatctacc

SEQ ID NO: 244 - DNA, 21 bp, Artificial Sequence
  LAG3-138
ccagctttccagctttcctct

SEQ ID NO: 245 - DNA, 21 bp, Artificial Sequence
  LAG3-503
gatctcagccttctgcgaaga

SEQ ID NO: 246 - DNA, 21 bp, Artificial Sequence
  LAG3-1092
gcttcaacgtctccatcatgt

SEQ ID NO: 247 - DNA, 21 bp, Artificial Sequence
  LAG3-1221
ggtctttcctcactgccaagt

SEQ ID NO: 248 - DNA, 21 bp, Artificial Sequence
  LAG3-1278
ctggagacaatggcgacttta

SEQ ID NO: 249 - DNA, 21 bp, Artificial Sequence
  LAG3-1379
gccactgtcacattggcaatc

SEQ ID NO: 250 - DNA, 21 bp, Artificial Sequence
  LAG3-1465
tccagtatctggacaagaacg

SEQ ID NO: 251 - DNA, 21 bp, Artificial Sequence
  LAG3-1616
gcagcagtgtacttcacagag

SEQ ID NO: 252 - DNA, 21 bp, Artificial Sequence
  LAG3-1702
gctgtttctcatccttggtgt

SEQ ID NO: 253 - DNA, 21 bp, Artificial Sequence
  LAG3-1751
gcctttggctttcacctttgg

SEQ ID NO: 254 - DNA, 21 bp, Artificial Sequence
  LAG3-1954
tcagcagcccagtccaaataa

SEQ ID NO: 255 - DNA, 21 bp, Artificial Sequence
  CTLA4-3
ggtggagctcatgtacccacc

SEQ ID NO: 256 - DNA, 21 bp, Artificial Sequence
  CTLA4-1
cccaaattacgtgtactacaa

SEQ ID NO: 257 - DNA, 21 bp, Artificial Sequence
  CTLA4-1058
gcatcacttgggattaatatg

SEQ ID NO: 258 - DNA, 21 bp, Artificial Sequence
  CTLA4-1154
gcgagggagaagactatattg

SEQ ID NO: 259 - DNA, 21 bp, Artificial Sequence
  CTLA4-1309
gccagtgatgctaaaggttgt

SEQ ID NO: 260 - DNA, 21 bp, Artificial Sequence
  CTLA4-1686
ggtggtatctgagttgacttg

SEQ ID NO: 261 - DNA, 21 bp, Artificial Sequence
  Tim3-1
gatgaaagggatgtgaattat

SEQ ID NO: 262 - DNA, 21 bp, Artificial Sequence
  Tim3-2
gggagcctccctgatataaat

SEQ ID NO: 263 - DNA, 19 bp, Artificial Sequence
  Tim3-3
ggaattcgctcagaagaaa

SEQ ID NO: 264 - DNA, 21 bp, Artificial Sequence
  Tim3-4
ggaccaaactgaagctatatt

SEQ ID NO: 265 - DNA, 21 bp, Artificial Sequence
  PD1-1
cctgtggttctattatattat

SEQ ID NO: 266 - DNA, 21 bp, Artificial Sequence
  PD1-2
gcctagagaagtttcagggaa

SEQ ID NO: 267 - DNA, 21 bp, Artificial Sequence
  PD1-3
cattgtctttcctagcggaat

SEQ ID NO: 268 - DNA, 20 bp, Artificial Sequence
  18s rRNA Forward
gattaagtccctgccctttg

SEQ ID NO: 269 - DNA, 20 bp, Artificial Sequence
  18s rRNA Reverse
gttcacctacggaaaccttg

SEQ ID NO: 270 - DNA, 20 bp, Artificial Sequence
  PDCD1 Forward
cctccacctttacacatgcc

SEQ ID NO: 271 - DNA, 20 bp, Artificial Sequence
  PDCD1 Reverse
cttactgcctcagcttccct

SEQ ID NO: 272 - DNA, 21 bp, Artificial Sequence
  IL2 Forward
ccaagaaggccacagaactga

SEQ ID NO: 273 - DNA, 26 bp, Artificial Sequence
  IL2 Reverse
gttgtttcagatccctttagttccag

SEQ ID NO: 274 - DNA, 21 bp, Artificial Sequence
  IL4 Forward
actttgaacagcctcacagag

SEQ ID NO: 275 - DNA, 22 bp, Artificial Sequence
  IL4 Reverse
ccgagttgaccgtaacagacat

SEQ ID NO: 276 - DNA, 20 bp, Artificial Sequence
  IL17A Forward
caaccgatccacctcacctt

SEQ ID NO: 277 - DNA, 19 bp, Artificial Sequence
  IL17A Reverse
ggcactttgcctcccagat

SEQ ID NO: 278 - DNA, 21 bp, Artificial Sequence
  CD25 Forward
cacaagctctgccactcggaa

SEQ ID NO: 279 - DNA, 20 bp, Artificial Sequence
  CD25 Reverse
tgcagtgacctggaaggctc

SEQ ID NO: 280 - DNA, 20 bp, Artificial Sequence
  CTLA4 Forward
ctacctgggcataggcaacg

SEQ ID NO: 281 - DNA, 20 bp, Artificial Sequence
  CTLA4 Reverse
ccccgaactaactgctgcaa

SEQ ID NO: 282 - DNA, 23 bp, Artificial Sequence
  FOXP3 Forward
gaaacagcacattcccagagttc

SEQ ID NO: 283 - DNA, 17 bp, Artificial Sequence
  FOXP3 Reverse
atggcccagcggatgag

SEQ ID NO: 284 - DNA, 19 bp, Artificial Sequence
  TGF-beta1 Forward
cccagcatctgcaaagctc

SEQ ID NO: 285 - DNA, 20 bp, Artificial Sequence
  TGF-beta1 Reverse
gtccttgcggaagtcaatgt

SEQ ID NO: 286 - DNA, 22 bp, Artificial Sequence
  TGFBR1 Forward
acatgattcagccacagatacc

SEQ ID NO: 287 - DNA, 21 bp, Artificial Sequence
  TGFBR1 Reverse
gcatagatgtcagcacgtttg

SEQ ID NO: 288 - DNA, 19 bp, Artificial Sequence
  TGFBR2 Forward
acgtgttgagagatcgagg

SEQ ID NO: 289 - DNA, 20 bp, Artificial Sequence
  TGFBR2 Reverse
cccagcactcagtcaacgtc

SEQ ID NO: 290 - DNA, 10 bp, Artificial Sequence
  NF-kB-RE 5x
gggaatttcc